European Patent Application EP 4 378 468 A1, published June 5, 2024. Title: A Composition for treating muscle loss related disease comprising Exosome derived from tonsil-mesenchymal stem cell. Applicant: Ewha University - Industry Collaboration Foundation. The sequence listing filed with the application follows.

SEQUENCE LISTING (15 sequences)

SEQ ID NO: 1 - RNA, 23 nt, Artificial Sequence
  hsa-miR-145-5p
guccaguuuucccaggaaucccu

SEQ ID NO: 2 - DNA, 21 bp, Artificial Sequence
  Murf1 Forward Primer
gtgtgaggtgcctacttgctc

SEQ ID NO: 3 - DNA, 21 bp, Artificial Sequence
  Murf1 Reverse Primer
tgagagatgatcgtctgcact

SEQ ID NO: 4 - DNA, 19 bp, Artificial Sequence
  Atrogin1 Forward Primer
cagcttcgtgagcgacctc

SEQ ID NO: 5 - DNA, 20 bp, Artificial Sequence
  Atrogin1 Reverse Primer
ggcagtcgagaagtccagtc

SEQ ID NO: 6 - DNA, 28 bp, Artificial Sequence
  Gapdh Forward Primer
ggtaaagtggatattgttgccatcaatg

SEQ ID NO: 7 - DNA, 28 bp, Artificial Sequence
  Gapdh Reverse Primer
ggagggatctcgctcctggaagatggtg

SEQ ID NO: 8 - DNA, 21 bp, Artificial Sequence
  MyoD Forward Primer
ccactccgggacatagacttg

SEQ ID NO: 9 - DNA, 20 bp, Artificial Sequence
  MyoD Reverse Primer
aaaagcgcaggtctggtgag

SEQ ID NO: 10 - DNA, 21 bp, Artificial Sequence
  Myh1 Forward Primer
gcgaatcgaggctcagaacaa

SEQ ID NO: 11 - DNA, 21 bp, Artificial Sequence
  Myh1 Reverse Primer
gtagttccgccttcggtcttg

SEQ ID NO: 12 - DNA, 22 bp, Artificial Sequence
  Acvr2a Forward Primer
ataaacggcgacattgttttgc

SEQ ID NO: 13 - DNA, 23 bp, Artificial Sequence
  Acvr2a Reverse Primer
tcggtgtaacaggatttgaagtg

SEQ ID NO: 14 - DNA, 22 bp, Artificial Sequence
  Acvr1b Forward Primer
ctgcctacagaccaactacacc

SEQ ID NO: 15 - DNA, 23 bp, Artificial Sequence
  Acvr1b Reverse Primer
gcagaagtcaatatagcagcagt